European Patent Specification EP 3 458 482 B1, published September 2, 2026. Title: ANTI-AXL TYROSINE KINASE RECEPTOR ANTIBODIES AND USES THEREOF. Applicant: AGENCY FOR SCIENCE, TECHNOLOGY AND RESEARCH. The sequence listing filed with the application follows.

SEQUENCE LISTING (15 sequences)

SEQ ID NO: 1 - protein, 119 aa, Artificial Sequence
  Isolated peptide sequence
QVKLQESGAELVKPGASVKLSCKASGFTFTSYYMYWVKQRPGQGLEWIGGVSPSNGGANFNEKFKTKATLTVDKSSSTAYMQLSSLTSEDSAVYYCTRFLYGPRYFDVWGQGTTVTVSS

SEQ ID NO: 2 - protein, 111 aa, Artificial Sequence
  Isolated peptide sequence
DIELTQSPASLAVSLGQRATISCRASESVDNYGISFMNWFQQKPGQPPKLLIYGASNQGSGVPARFSGSGSGTDFSLNIHPMEEDDTAMYFCQQSKEVPYTFGGGTKLEIK

SEQ ID NO: 3 - protein, 10 aa, Artificial Sequence
  Isolated peptide sequence
GFTFTSYYMY

SEQ ID NO: 4 - protein, 17 aa, Artificial Sequence
  Isolated peptide sequence
GVSPSNGGANFNEKFKT

SEQ ID NO: 5 - protein, 10 aa, Artificial Sequence
  Isolated peptide sequence
FLYGPRYFDV

SEQ ID NO: 6 - protein, 15 aa, Artificial Sequence
  Isolated peptide sequence
RASESVDNYGISFMN

SEQ ID NO: 7 - protein, 7 aa, Artificial Sequence
  Isolated peptide sequence
GASNQGS

SEQ ID NO: 8 - protein, 9 aa, Artificial Sequence
  Isolated peptide sequence
QQSKEVPYT

SEQ ID NO: 9 - DNA, 20 bp, Artificial Sequence
  Primer sequence
ggtggctgtgaagacgatga

SEQ ID NO: 10 - DNA, 20 bp, Artificial Sequence
  Primer sequence
ctcagatactccatgccact

SEQ ID NO: 11 - DNA, 21 bp, Artificial Sequence
  siRNA sequence
cagcgagauuuaugacuautt

SEQ ID NO: 12 - DNA, 357 bp, Artificial Sequence
  Isolated genetic sequence
caggtcaaactgcaggagtcaggggctgaactggtgaagcctggggcttcagtgaagttgtcctgtaaggcttctggcttcaccttcaccagctactatatgtactgggtgaagcagaggcctggacaaggccttgagtggattgggggggttagtcctagcaatggtggtgctaacttcaatgagaagttcaagaccaaggccacactgactgtagacaaatcctccagcacagcctacatgcaactcagcagcctgacatctgaggactctgcggtctattactgtacaagattcctttatggtccgaggtacttcgatgtctggggccaagggaccacggtcaccgtctcctca

SEQ ID NO: 13 - DNA, 334 bp, Artificial Sequence
  Isolated genetic sequence
gacattgagctcacccagtctccagcttctttggctgtgtctctagggcagagggccaccatctcctgcagagccagcgaaagtgttgataattatggcattagttttatgaactggttccaacagaaaccaggacagccacccaaactcctcatttatggtgcatccaaccagggatccggggtccctgccaggtttagtggcagtgggtctgggacagacttcagcctcaacatccatcctatggaggaggatgatactgcaatgtatttctgtcagcaaagtaaggaggttccgtacacgttcggaggggggaccaagctggaaataaaac

SEQ ID NO: 14 - protein, 894 aa, Homo sapiens
MAWRCPRMGRVPLAWCLALCGWACMAPRGTQAEESPFVGNPGNITGARGLTGTLRCQLQVQGEPPEVHWLRDGQILELADSTQTQVPLGEDEQDDWIVVSQLRITSLQLSDTGQYQCLVFLGHQTFVSQPGYVGLEGLPYFLEEPEDRTVAANTPFNLSCQAQGPPEPVDLLWLQDAVPLATAPGHGPQRSLHVPGLNKTSSFSCEAHNAKGVTTSRTATITVLPQQPRNLHLVSRQPTELEVAWTPGLSGIYPLTHCTLQAVLSNDGMGIQAGEPDPPEEPLTSQASVPPHQLRLGSLHPHTPYHIRVACTSSQGPSSWTHWLPVETPEGVPLGPPENISATRNGSQAFVHWQEPRAPLQGTLLGYRLAYQGQDTPEVLMDIGLRQEVTLELQGDGSVSNLTVCVAAYTAAGDGPWSLPVPLEAWRPGQAQPVHQLVKEPSTPAFSWPWWYVLLGAVVAAACVLILALFLVHRRKKETRYGEVFEPTVERGELVVRYRVRKSYSRRTTEATLNSLGISEELKEKLRDVMVDRHKVALGKTLGEGEFGAVMEGQLNQDDSILKVAVKTMKIAICTRSELEDFLSEAVCMKEFDHPNVMRLIGVCFQGSERESFPAPVVILPFMKHGDLHSFLLYSRLGDQPVYLPTQMLVKFMADIASGMEYLSTKRFIHRDLAARNCMLNENMSVCVADFGLSKKIYNGDYYRQGRIAKMPVKWIAIESLADRVYTSKSDVWSFGVTMWEIATRGQTPYPGVENSEIYDYLRQGNRLKQPADCLDGLYALMSRCWELNPQDRPSFTELREDLENTLKALPPAQEPDEILYVNMDEGGGYPEPPGAAGGADPPTQPDPKDSCSCLTAAEVHPAGRYVLCPSTTPSPAQPADRGSPAAPGQEDGA

SEQ ID NO: 15 - protein, 894 aa, Homo sapiens; identical to SEQ ID NO: 14